European Patent Application EP 4 796 566 A1, published August 26, 2026. Title: ＡＡＶのキャプシドと標的受容体に同時に結合することができる分子. Applicant: 大阪大学. The sequence listing filed with the application follows.

SEQUENCE LISTING (54 sequences)

SEQ ID NO: 1 - protein, 13 aa, synthetic construct
YTYRTTIPHEYLA

SEQ ID NO: 2 - protein, 10 aa, synthetic construct
YSKSVCLAQD

SEQ ID NO: 3 - protein, 10 aa, synthetic construct
FSKSLHLAQE

SEQ ID NO: 4 - protein, 12 aa, synthetic construct
TYRTTIPHEYLA

SEQ ID NO: 5 - protein, 12 aa, synthetic construct
TYRTTIPNEYLA

SEQ ID NO: 6 - protein, 12 aa, synthetic construct
TYRTTIHHEYLA

SEQ ID NO: 7 - protein, 12 aa, synthetic construct
TYRTTIPHEYIA

SEQ ID NO: 8 - protein, 12 aa, synthetic construct
TYRTTITHEYLA

SEQ ID NO: 9 - protein, 4 aa, synthetic construct
SKSV

SEQ ID NO: 10 - protein, 4 aa, synthetic construct
TKST

SEQ ID NO: 11 - protein, 4 aa, synthetic construct
SKSI

SEQ ID NO: 12 - protein, 4 aa, synthetic construct
SKSA

SEQ ID NO: 13 - protein, 4 aa, synthetic construct
SKRV

SEQ ID NO: 14 - protein, 9 aa, synthetic construct
LAQDWEYKW

SEQ ID NO: 15 - protein, 8 aa, synthetic construct
LAQDWEYK

SEQ ID NO: 16 - protein, 9 aa, synthetic construct
LAKDWEYKW

SEQ ID NO: 17 - protein, 9 aa, synthetic construct
LAQDWVYKY

SEQ ID NO: 18 - protein, 9 aa, synthetic construct
LAQDWKYKW

SEQ ID NO: 19 - protein, 15 aa, synthetic construct
RFSKSLHLAQQYQRI

SEQ ID NO: 20 - protein, 15 aa, synthetic construct
RFSKSLHLAQEYQRI

SEQ ID NO: 21 - protein, 15 aa, synthetic construct
RFSKSLHLAQQYQQI

SEQ ID NO: 22 - protein, 15 aa, synthetic construct
RFSKSLHLAQQYKRI

SEQ ID NO: 23 - protein, 15 aa, synthetic construct
RFSKSLHLAQQYQLI

SEQ ID NO: 24 - protein, 12 aa, synthetic construct
TYRTTIPHEYLD

SEQ ID NO: 25 - protein, 12 aa, synthetic construct
TYSTTIPHEYLA

SEQ ID NO: 26 - protein, 12 aa, synthetic construct
TYRTTIPYEYLA

SEQ ID NO: 27 - protein, 12 aa, synthetic construct
TYHTTIPHEYLA

SEQ ID NO: 28 - protein, 12 aa, synthetic construct
TYRNTIPHEYLA

SEQ ID NO: 29 - protein, 12 aa, synthetic construct
NYRTTIPHEYLA

SEQ ID NO: 30 - protein, 12 aa, synthetic construct
IYRTTIPHEYLA

SEQ ID NO: 31 - protein, 12 aa, synthetic construct
TYRTTIPPEYLA

SEQ ID NO: 32 - protein, 12 aa, synthetic construct
TYRTTIPHEYLV

SEQ ID NO: 33 - protein, 12 aa, synthetic construct
TYRTTIPHEYLT

SEQ ID NO: 34 - protein, 9 aa, synthetic construct
LAQDWEYEW

SEQ ID NO: 35 - protein, 9 aa, synthetic construct
LAQDWEYLA

SEQ ID NO: 36 - protein, 9 aa, synthetic construct
LAQDWEYRW

SEQ ID NO: 37 - protein, 9 aa, synthetic construct
LAQNWEYKW

SEQ ID NO: 38 - protein, 9 aa, synthetic construct
LAQDWDYKW

SEQ ID NO: 39 - protein, 8 aa, synthetic construct
LAKDWEYK

SEQ ID NO: 40 - protein, 9 aa, synthetic construct
LTQDWEYKW

SEQ ID NO: 41 - protein, 9 aa, synthetic construct
LAQDWEYNW

SEQ ID NO: 42 - protein, 9 aa, synthetic construct
LAQDWEYKW

SEQ ID NO: 43 - protein, 9 aa, synthetic construct
LAQDWEYKR

SEQ ID NO: 44 - protein, 15 aa, synthetic construct
RFYKSLHLAQQYQRI

SEQ ID NO: 45 - protein, 15 aa, synthetic construct
RFSKSLHIAQQYQRI

SEQ ID NO: 46 - protein, 15 aa, synthetic construct
RFSKSFHLAQQYQRI

SEQ ID NO: 47 - protein, 22 aa, synthetic construct
SGGGCYTYRTTIPHEYLCGGGS

SEQ ID NO: 48 - protein, 30 aa, synthetic construct
SGGGSGCYRFSKSLHLAQEYQRICGGSGGS

SEQ ID NO: 49 - protein, 18 aa, synthetic construct
SGWRPRVARWTGQIIYGS

SEQ ID NO: 50 - protein, 23 aa, synthetic construct
SGGCASFPEELDEWYVAYGCGGS

SEQ ID NO: 51 - protein, 21 aa, synthetic construct
SGGYVEPIVTRYAIYWKLGGS

SEQ ID NO: 52 - protein, 15 aa, synthetic construct
SGCYLRPRYKFWCGS

SEQ ID NO: 53 - protein, 19 aa, synthetic construct
SGGYTGHTWTLNSGYRGGS

SEQ ID NO: 54 - protein, 22 aa, synthetic construct
SGGGCYTYRNTIPHEYLCGGGS